European Patent Application EP 4 512 892 A1, published February 26, 2025. Title: Glycoprotein with reduced number of mannose-6-phosphate. Applicant: JCR Pharmaceuticals Co., Ltd. The sequence listing filed with the application follows.

SEQUENCE LISTING (42 sequences)

SEQ ID NO: 1 - protein, 525 aa, Homo sapiens
SETQANSTTDALNVLLIIVDDLRPSLGCYGDKLVRSPNIDQLASHSLLFQNAFAQQAVCAPSRVSFLTGRRPDTTRLYDFNSYWRVHAGNFSTIPQYFKENGYVTMSVGKVFHPGISSNHTDDSPYSWSFPPYHPSSEKYENTKTCRGPDGELHANLLCPVDVLDVPEGTLPDKQSTEQAIQLLEKMKTSASPFFLAVGYHKPHIPFRYPKEFQKLYPLENITLAPDPEVPDGLPPVAYNPWMDIRQREDVQALNISVPYGPIPVDFQRKIRQSYFASVSYLDTQVGRLLSALDDLQLANSTIIAFTSDHGWALGEHGEWAKYSNFDVATHVPLIFYVPGRTASLPEAGEKLFPYLDPFDSASQLMEPGRQSMDLVELVSLFPTLAGLAGLQVPPRCPVPSFHVELCREGKNLLKHFRFRDLEEDPYLPGNPRELIAYSQYPRPSDIPQWNSDKPSLKDIKIMGYSIRTIDYRYTVWVGFNPDEFLANFSDIHAGELYFVDSDPLQDHNMYNDSQGGDLFQLLMP

SEQ ID NO: 2 - DNA, 1575 bp, Homo sapiens
  source 1..1575: mol_type = genomic DNA
tccgaaacgcaggccaactcgaccacagatgctctgaacgttcttctcatcatcgtggatgacctgcgcccctccctgggctgttatggggataagctggtgaggtccccaaatattgaccaactggcatcccacagcctcctcttccagaatgcctttgcgcagcaagcagtgtgcgccccgagccgcgtttctttcctcactggcaggagacctgacaccacccgcctgtacgacttcaactcctactggagggtgcacgctggaaacttctccaccatcccccagtacttcaaggagaatggctatgtgaccatgtcggtgggaaaagtctttcaccctgggatatcttctaaccataccgatgattctccgtatagctggtcttttccaccttatcatccttcctctgagaagtatgaaaacactaagacatgtcgagggccagatggagaactccatgccaacctgctttgccctgtggatgtgctggatgttcccgagggcaccttgcctgacaaacagagcactgagcaagccatacagttgttggaaaagatgaaaacgtcagccagtcctttcttcctggccgttgggtatcataagccacacatccccttcagataccccaaggaatttcagaagttgtatcccttggagaacatcaccctggcccccgatcccgaggtccctgatggcctaccccctgtggcctacaacccctggatggacatcaggcaacgggaagacgtccaagccttaaacatcagtgtgccgtatggtccaattcctgtggactttcagcggaaaatccgccagagctactttgcctctgtgtcatatttggatacacaggtcggccgcctcttgagtgctttggacgatcttcagctggccaacagcaccatcattgcatttacctcggatcatgggtgggctctaggtgaacatggagaatgggccaaatacagcaattttgatgttgctacccatgttcccctgatattctatgttcctggaaggacggcttcacttccggaggcaggcgagaagcttttcccttacctcgacccttttgattccgcctcacagttgatggagccaggcaggcaatccatggaccttgtggaacttgtgtctctttttcccacgctggctggacttgcaggactgcaggttccacctcgctgccccgttccttcatttcacgttgagctgtgcagagaaggcaagaaccttctgaagcattttcgattccgtgacttggaagaagatccgtacctccctggtaatccccgtgaactgattgcctatagccagtatccccggccttcagacatccctcagtggaattctgacaagccgagtttaaaagatataaagatcatgggctattccatacgcaccatagactataggtatactgtgtgggttggcttcaatcctgatgaatttctagctaacttttctgacatccatgcaggggaactgtattttgtggattctgacccattgcaggatcacaatatgtataatgattcccaaggtggagaccttttccagttgttgatgcct

SEQ ID NO: 3 - protein, 550 aa, Homo sapiens
MPPPRTGRGLLWLGLVLSSVCVALGSETQANSTTDALNVLLIIVDDLRPSLGCYGDKLVRSPNIDQLASHSLLFQNAFAQQAVCAPSRVSFLTGRRPDTTRLYDFNSYWRVHAGNFSTIPQYFKENGYVTMSVGKVFHPGISSNHTDDSPYSWSFPPYHPSSEKYENTKTCRGPDGELHANLLCPVDVLDVPEGTLPDKQSTEQAIQLLEKMKTSASPFFLAVGYHKPHIPFRYPKEFQKLYPLENITLAPDPEVPDGLPPVAYNPWMDIRQREDVQALNISVPYGPIPVDFQRKIRQSYFASVSYLDTQVGRLLSALDDLQLANSTIIAFTSDHGWALGEHGEWAKYSNFDVATHVPLIFYVPGRTASLPEAGEKLFPYLDPFDSASQLMEPGRQSMDLVELVSLFPTLAGLAGLQVPPRCPVPSFHVELCREGKNLLKHFRFRDLEEDPYLPGNPRELIAYSQYPRPSDIPQWNSDKPSLKDIKIMGYSIRTIDYRYTVWVGFNPDEFLANFSDIHAGELYFVDSDPLQDHNMYNDSQGGDLFQLLMP

SEQ ID NO: 4 - protein, 525 aa, synthetic construct
  REGION 1..525: note = amino acid sequence of lightly M6P-glycosylated type hIDS 1(amino acid sequence of muhIDS-2)
SETQANSTTDALNVLLIIVDDLRPSLGCYGDKLVRSPNIDQLASHSLLFQNAFAQQAVCAPSRVSFLTGRRPDTTRLYDFNSYWRVHAGNFSTIPQYFKENGYVTMSVGKVFHPGISSNHTDDSPYSWSFPPYHPSSEKYENTKTCRGPDGELHANLLCPVDVLDVPEGTLPDKQSTEQAIQLLEKMKTSASPFFLAVGYHKPHIPFRYPKEFQKLYPLEQITLAPDPEVPDGLPPVAYNPWMDIRQREDVQALQISVPYGPIPVDFQRKIRQSYFASVSYLDTQVGRLLSALDDLQLANSTIIAFTSDHGWALGEHGEWAKYSNFDVATHVPLIFYVPGRTASLPEAGEKLFPYLDPFDSASQLMEPGRQSMDLVELVSLFPTLAGLAGLQVPPRCPVPSFHVELCREGKNLLKHFRFRDLEEDPYLPGNPRELIAYSQYPRPSDIPQWNSDKPSLKDIKIMGYSIRTIDYRYTVWVGFNPDEFLANFSDIHAGELYFVDSDPLQDHNMYNDSQGGDLFQLLMP

SEQ ID NO: 5 - protein, 525 aa, synthetic construct
  REGION 1..525: note = amino acid sequence of lightly M6P-glycosylated type hIDS 2(amino acid sequence of muhIDS-1)
SETQANSTTDALNVLLIIVDDLRPSLGCYGDKLVRSPNIDQLASHSLLFQNAFAQQAVCAPSRVSFLTGRRPDTTRLYDFNSYWRVHAGNFSTIPQYFKENGYVTMSVGKVFHPGISSNHTDDSPYSWSFPPYHPSSEKYENTKTCRGPDGELHANLLCPVDVLDVPEGTLPDKQSTEQAIQLLEKMKTSASPFFLAVGYHKPHIPFRYPKEFQKLYPLENIALAPDPEVPDGLPPVAYNPWMDIRQREDVQALNIAVPYGPIPVDFQRKIRQSYFASVSYLDTQVGRLLSALDDLQLANSTIIAFTSDHGWALGEHGEWAKYSNFDVATHVPLIFYVPGRTASLPEAGEKLFPYLDPFDSASQLMEPGRQSMDLVELVSLFPTLAGLAGLQVPPRCPVPSFHVELCREGKNLLKHFRFRDLEEDPYLPGNPRELIAYSQYPRPSDIPQWNSDKPSLKDIKIMGYSIRTIDYRYTVWVGFNPDEFLANFSDIHAGELYFVDSDPLQDHNMYNDSQGGDLFQLLMP

SEQ ID NO: 6 - protein, 525 aa, synthetic construct
  REGION 1..525: note = amino acid sequence of lightly M6P-glycosylated type hIDS 3
SETQANSTTDALNVLLIIVDDLRPSLGCYGDKLVRSPNIDQLASHSLLFQNAFAQQAVCAPSRVSFLTGRRPDTTRLYDFNSYWRVHAGNFSTIPQYFKENGYVTMSVGKVFHPGISSNHTDDSPYSWSFPPYHPSSEKYENTKTCRGPDGELHANLLCPVDVLDVPEGTLPDKQSTEQAIQLLEKMKTSASPFFLAVGYHKPHIPFRYPKEFQKLYPLEQIALAPDPEVPDGLPPVAYNPWMDIRQREDVQALQIAVPYGPIPVDFQRKIRQSYFASVSYLDTQVGRLLSALDDLQLANSTIIAFTSDHGWALGEHGEWAKYSNFDVATHVPLIFYVPGRTASLPEAGEKLFPYLDPFDSASQLMEPGRQSMDLVELVSLFPTLAGLAGLQVPPRCPVPSFHVELCREGKNLLKHFRFRDLEEDPYLPGNPRELIAYSQYPRPSDIPQWNSDKPSLKDIKIMGYSIRTIDYRYTVWVGFNPDEFLANFSDIHAGELYFVDSDPLQDHNMYNDSQGGDLFQLLMP

SEQ ID NO: 7 - protein, 628 aa, Homo sapiens
AEAPHLVHVDAARALWPLRRFWRSTGFCPPLPHSQADQYVLSWDQQLNLAYVGAVPHRGIKQVRTHWLLELVTTRGSTGRGLSYNFTHLDGYLDLLRENQLLPGFELMGSASGHFTDFEDKQQVFEWKDLVSSLARRYIGRYGLAHVSKWNFETWNEPDHHDFDNVSMTMQGFLNYYDACSEGLRAASPALRLGGPGDSFHTPPRSPLSWGLLRHCHDGTNFFTGEAGVRLDYISLHRKGARSSISILEQEKVVAQQIRQLFPKFADTPIYNDEADPLVGWSLPQPWRADVTYAAMVVKVIAQHQNLLLANTTSAFPYALLSNDNAFLSYHPHPFAQRTLTARFQVNNTRPPHVQLLRKPVLTAMGLLALLDEEQLWAEVSQAGTVLDSNHTVGVLASAHRPQGPADAWRAAVLIYASDDTRAHPNRSVAVTLRLRGVPPGPGLVYVTRYLDNGLCSPDGEWRRLGRPVFPTAEQFRRMRAAEDPVAAAPRPLPAGGRLTLRPALRLPSLLLVHVCARPEKPPGQVTRLRALPLTQGQLVLVWSDEHVGSKCLWTYEIQFSQDGKAYTPVSRKPSTFNLFVFSPDTGAVSGSYRVRALDYWARPGPFSDPVPYLEVPVPRGPPSPGNP

SEQ ID NO: 8 - DNA, 1885 bp, Homo sapiens
  source 1..1885: mol_type = genomic DNA
tgccgaggccccgcacctggtgcacgtggacgcggcccgcgcgctgtggcccctgcggcgcttctggaggagcacaggcttctgccccccgctgccacacagccaggctgaccagtacgtcctcagctgggaccagcagctcaacctcgcctatgtgggcgccgtccctcaccgcggcatcaagcaggtccggacccactggctgctggagcttgtcaccaccagggggtccactggacggggcctgagctacaacttcacccacctggacgggtacttggaccttctcagggagaaccagctcctcccagggtttgagctgatgggcagcgcctcgggccacttcactgactttgaggacaagcagcaggtgtttgagtggaaggacttggtctccagcctggccaggagatacatcggtaggtacggactggcgcatgtttccaagtggaacttcgagacgtggaatgagccagaccaccacgactttgacaacgtctccatgaccatgcaaggcttcctgaactactacgatgcctgctcggagggtctgcgcgccgccagccccgccctgcggctgggaggccccggcgactccttccacaccccaccgcgatccccgctgagctggggcctcctgcgccactgccacgacggtaccaacttcttcactggggaggcgggcgtgcggctggactacatctccctccacaggaagggtgcgcgcagctccatctccatcctggagcaggagaaggtcgtcgcgcagcagatccggcagctcttccccaagttcgcggacacccccatttacaacgacgaggcggacccgctggtgggctggtccctgccacagccgtggagggcggacgtgacctacgcggccatggtggtgaaggtcatcgcgcagcatcagaacctgctactggccaacaccacctccgccttcccctacgcgctcctgagcaacgacaatgccttcctgagctaccacccgcaccccttcgcgcagcgcacgctcaccgcgcgcttccaggtcaacaacacccgcccgccgcacgtgcagctgttgcgcaagccggtgctcacggccatggggctgctggcgctgctggatgaggagcagctctgggccgaagtgtcgcaggccgggaccgtcctggacagcaaccacacggtgggcgtcctggccagcgcccaccgcccccagggcccggccgacgcctggcgcgccgcggtgctgatctacgcgagcgacgacacccgcgcccaccccaaccgcagcgtcgcggtgaccctgcggctgcgcggggtgccccccggcccgggcctggtctacgtcacgcgctacctggacaacgggctctgcagccccgacggcgagtggcggcgcctgggccggcccgtcttccccacggcagagcagttccggcgcatgcgcgcggctgaggacccggtggccgcggcgccccgccccttacccgccggtggccgcctgaccctgcgccccgcgctgcggctgccgtcgcttttgctggtgcacgtgtgtgcgcgccccgagaagccgcccgggcaggtcacgcggctccgcgccctgcccctgacccaagggcagctggttctggtctggtcggatgaacacgtgggctccaagtgcctgtggacatacgagatccagttctctcaggacggtaaggcgtacaccccggtcagcaggaagccatcgaccttcaacctctttgtgttcagcccagacacaggtgctgtctctggctcctaccgagttcgagccctggactactgggcccgaccaggccccttctcggaccctgtgccgtacctggaggtccctgtgccaagagggcccccatccccgggcaatcca

SEQ ID NO: 9 - protein, 653 aa, Homo sapiens
MRPLRPRAALLALLASLLAAPPVAPAEAPHLVHVDAARALWPLRRFWRSTGFCPPLPHSQADQYVLSWDQQLNLAYVGAVPHRGIKQVRTHWLLELVTTRGSTGRGLSYNFTHLDGYLDLLRENQLLPGFELMGSASGHFTDFEDKQQVFEWKDLVSSLARRYIGRYGLAHVSKWNFETWNEPDHHDFDNVSMTMQGFLNYYDACSEGLRAASPALRLGGPGDSFHTPPRSPLSWGLLRHCHDGTNFFTGEAGVRLDYISLHRKGARSSISILEQEKVVAQQIRQLFPKFADTPIYNDEADPLVGWSLPQPWRADVTYAAMVVKVIAQHQNLLLANTTSAFPYALLSNDNAFLSYHPHPFAQRTLTARFQVNNTRPPHVQLLRKPVLTAMGLLALLDEEQLWAEVSQAGTVLDSNHTVGVLASAHRPQGPADAWRAAVLIYASDDTRAHPNRSVAVTLRLRGVPPGPGLVYVTRYLDNGLCSPDGEWRRLGRPVFPTAEQFRRMRAAEDPVAAAPRPLPAGGRLTLRPALRLPSLLLVHVCARPEKPPGQVTRLRALPLTQGQLVLVWSDEHVGSKCLWTYEIQFSQDGKAYTPVSRKPSTFNLFVFSPDTGAVSGSYRVRALDYWARPGPFSDPVPYLEVPVPRGPPSPGNP

SEQ ID NO: 10 - protein, 628 aa, synthetic construct
  REGION 1..628: note = amino acid sequence of lightly M6P-glycosylated type hIDUA 1
AEAPHLVHVDAARALWPLRRFWRSTGFCPPLPHSQADQYVLSWDQQLNLAYVGAVPHRGIKQVRTHWLLELVTTRGSTGRGLSYNFTHLDGYLDLLRENQLLPGFELMGSASGHFTDFEDKQQVFEWKDLVSSLARRYIGRYGLAHVSKWNFETWNEPDHHDFDNVSMTMQGFLNYYDACSEGLRAASPALRLGGPGDSFHTPPRSPLSWGLLRHCHDGTNFFTGEAGVRLDYISLHRKGARSSISILEQEKVVAQQIRQLFPKFADTPIYNDEADPLVGWSLPQPWRADVTYAAMVVKVIAQHQNLLLAQTTSAFPYALLSNDNAFLSYHPHPFAQRTLTARFQVNNTRPPHVQLLRKPVLTAMGLLALLDEEQLWAEVSQAGTVLDSNHTVGVLASAHRPQGPADAWRAAVLIYASDDTRAHPQRSVAVTLRLRGVPPGPGLVYVTRYLDNGLCSPDGEWRRLGRPVFPTAEQFRRMRAAEDPVAAAPRPLPAGGRLTLRPALRLPSLLLVHVCARPEKPPGQVTRLRALPLTQGQLVLVWSDEHVGSKCLWTYEIQFSQDGKAYTPVSRKPSTFNLFVFSPDTGAVSGSYRVRALDYWARPGPFSDPVPYLEVPVPRGPPSPGNP

SEQ ID NO: 11 - protein, 628 aa, synthetic construct
  REGION 1..628: note = amino acid sequence of lightly M6P-glycosylated type hIDUA 2
AEAPHLVHVDAARALWPLRRFWRSTGFCPPLPHSQADQYVLSWDQQLNLAYVGAVPHRGIKQVRTHWLLELVTTRGSTGRGLSYNFTHLDGYLDLLRENQLLPGFELMGSASGHFTDFEDKQQVFEWKDLVSSLARRYIGRYGLAHVSKWNFETWNEPDHHDFDNVSMTMQGFLNYYDACSEGLRAASPALRLGGPGDSFHTPPRSPLSWGLLRHCHDGTNFFTGEAGVRLDYISLHRKGARSSISILEQEKVVAQQIRQLFPKFADTPIYNDEADPLVGWSLPQPWRADVTYAAMVVKVIAQHQNLLLANTASAFPYALLSNDNAFLSYHPHPFAQRTLTARFQVNNTRPPHVQLLRKPVLTAMGLLALLDEEQLWAEVSQAGTVLDSNHTVGVLASAHRPQGPADAWRAAVLIYASDDTRAHPNRAVAVTLRLRGVPPGPGLVYVTRYLDNGLCSPDGEWRRLGRPVFPTAEQFRRMRAAEDPVAAAPRPLPAGGRLTLRPALRLPSLLLVHVCARPEKPPGQVTRLRALPLTQGQLVLVWSDEHVGSKCLWTYEIQFSQDGKAYTPVSRKPSTFNLFVFSPDTGAVSGSYRVRALDYWARPGPFSDPVPYLEVPVPRGPPSPGNP

SEQ ID NO: 12 - protein, 628 aa, synthetic construct
  REGION 1..628: note = amino acid sequence of lightly M6P-glycosylated type hIDUA 3
AEAPHLVHVDAARALWPLRRFWRSTGFCPPLPHSQADQYVLSWDQQLNLAYVGAVPHRGIKQVRTHWLLELVTTRGSTGRGLSYNFTHLDGYLDLLRENQLLPGFELMGSASGHFTDFEDKQQVFEWKDLVSSLARRYIGRYGLAHVSKWNFETWNEPDHHDFDNVSMTMQGFLNYYDACSEGLRAASPALRLGGPGDSFHTPPRSPLSWGLLRHCHDGTNFFTGEAGVRLDYISLHRKGARSSISILEQEKVVAQQIRQLFPKFADTPIYNDEADPLVGWSLPQPWRADVTYAAMVVKVIAQHQNLLLAQTASAFPYALLSNDNAFLSYHPHPFAQRTLTARFQVNNTRPPHVQLLRKPVLTAMGLLALLDEEQLWAEVSQAGTVLDSNHTVGVLASAHRPQGPADAWRAAVLIYASDDTRAHPQRAVAVTLRLRGVPPGPGLVYVTRYLDNGLCSPDGEWRRLGRPVFPTAEQFRRMRAAEDPVAAAPRPLPAGGRLTLRPALRLPSLLLVHVCARPEKPPGQVTRLRALPLTQGQLVLVWSDEHVGSKCLWTYEIQFSQDGKAYTPVSRKPSTFNLFVFSPDTGAVSGSYRVRALDYWARPGPFSDPVPYLEVPVPRGPPSPGNP

SEQ ID NO: 13 - protein, 482 aa, Homo sapiens
RPRNALLLLADDGGFESGAYNNSAIATPHLDALARRSLLFRNAFTSVSSCSPSRASLLTGLPQHQNGMYGLHQDVHHFNSFDKVRSLPLLLSQAGVRTGIIGKKHVGPETVYPFDFAYTEENGSVLQVGRNITRIKLLVRKFLQTQDDRPFFLYVAFHDPHRCGHSQPQYGTFCEKFGNGESGMGRIPDWTPQAYDPLDVLVPYFVPNTPAARADLAAQYTTVGRMDQGVGLVLQELRDAGVLNDTLVIFTSDNGIPFPSGRTNLYWPGTAEPLLVSSPEHPKRWGQVSEAYVSLLDLTPTILDWFSIPYPSYAIFGSKTIHLTGRSLLPALEAEPLWATVFGSQSHHEVTMSYPMRSVQHRHFRLVHNLNFKMPFPIDQDFYVSPTFQDLLNRTTAGQPTGWYKDLRHYYYRARWELYDRSRDPHETQNLATDPRFAQLLEMLRDQLAKWQWETHDPWVCAPDGVLEEKLSPQCQPLHNEL

SEQ ID NO: 14 - DNA, 1449 bp, Homo sapiens
  source 1..1449: mol_type = genomic DNA
cgtcctaggaatgctttattattactcgccgatgacggcggattcgagagcggagcctacaacaacagcgccatcgccaccccccatctggatgctctggctcgtcggtctttactctttcgtaacgctttcacatccgtcagctcttgtagcccttctcgtgcctctttactgactggtttaccccagcaccagaacggcatgtacggcctccaccaagacgtgcaccacttcaacagcttcgacaaggtgaggtctttacctctgctgctgagccaagctggagtgcggaccggcatcattggcaagaagcatgtgggccccgaaaccgtgtacccctttgatttcgcctacaccgaggaaaacggctccgtgctgcaagttggacggaatatcactcgtatcaagttattagtgcggaagttcctccagacccaagatgataggcccttctttttatacgtggctttccacgaccctcataggtgcggccactcccagccccagtatggcaccttctgcgagaagttcggcaacggcgaatccggaatgggtcgtatccccgattggacacctcaagcttacgaccctctggatgtgctggtgccctacttcgtgcctaacacccccgctgcccgggctgatctggctgctcagtatacaaccgtgggtcgtatggatcaaggtgtcggactggtgctgcaagaactgagggacgccggcgtgctcaacgacacactggtgatcttcacctccgacaacggcatccccttccccagcggaaggaccaatttatactggcccggtacagccgagcctctgctcgtgtcctcccccgaacaccccaagcggtggggacaagttagcgaagcttacgtctctttactggatctcacccccaccatcctcgattggtttagcatcccctatcccagctacgccatctttggcagcaagacaatccacctcactggtaggtctttactgcccgctttagaggctgagcctttatgggctaccgtcttcggctcccagtcccatcacgaagtcacaatgtcctaccccatgaggagcgtgcagcatcgtcacttccggctcgtccacaatctgaacttcaagatgcctttccccatcgaccaagatttctacgtgagccctaccttccaagatctcctcaatcggaccaccgctggccaacccaccggatggtacaaggatctgcggcactactactaccgggctcgttgggagctgtatgatcgttctcgtgatccccatgaaacccagaatctggccaccgacccccggtttgctcagctgctcgagatgttacgtgatcagctggccaagtggcagtgggagacacacgacccttgggtgtgcgctcccgatggcgtgctggaagagaaactgagccctcagtgccagcctctgcacaatgagctgtga

SEQ ID NO: 15 - protein, 502 aa, Homo sapiens
MSCPVPACCALLLVLGLCRARPRNALLLLADDGGFESGAYNNSAIATPHLDALARRSLLFRNAFTSVSSCSPSRASLLTGLPQHQNGMYGLHQDVHHFNSFDKVRSLPLLLSQAGVRTGIIGKKHVGPETVYPFDFAYTEENGSVLQVGRNITRIKLLVRKFLQTQDDRPFFLYVAFHDPHRCGHSQPQYGTFCEKFGNGESGMGRIPDWTPQAYDPLDVLVPYFVPNTPAARADLAAQYTTVGRMDQGVGLVLQELRDAGVLNDTLVIFTSDNGIPFPSGRTNLYWPGTAEPLLVSSPEHPKRWGQVSEAYVSLLDLTPTILDWFSIPYPSYAIFGSKTIHLTGRSLLPALEAEPLWATVFGSQSHHEVTMSYPMRSVQHRHFRLVHNLNFKMPFPIDQDFYVSPTFQDLLNRTTAGQPTGWYKDLRHYYYRARWELYDRSRDPHETQNLATDPRFAQLLEMLRDQLAKWQWETHDPWVCAPDGVLEEKLSPQCQPLHNEL

SEQ ID NO: 16 - protein, 482 aa, synthetic construct
  REGION 1..482: note = amino acid sequence of lightly M6P-glycosylated type hSGSH 1
RPRNALLLLADDGGFESGAYNNSAIATPHLDALARRSLLFRNAFTSVSSCSPSRASLLTGLPQHQNGMYGLHQDVHHFNSFDKVRSLPLLLSQAGVRTGIIGKKHVGPETVYPFDFAYTEENGSVLQVGRNITRIKLLVRKFLQTQDDRPFFLYVAFHDPHRCGHSQPQYGTFCEKFGNGESGMGRIPDWTPQAYDPLDVLVPYFVPNTPAARADLAAQYTTVGRMDQGVGLVLQELRDAGVLQDTLVIFTSDNGIPFPSGRTNLYWPGTAEPLLVSSPEHPKRWGQVSEAYVSLLDLTPTILDWFSIPYPSYAIFGSKTIHLTGRSLLPALEAEPLWATVFGSQSHHEVTMSYPMRSVQHRHFRLVHNLNFKMPFPIDQDFYVSPTFQDLLNRTTAGQPTGWYKDLRHYYYRARWELYDRSRDPHETQNLATDPRFAQLLEMLRDQLAKWQWETHDPWVCAPDGVLEEKLSPQCQPLHNEL

SEQ ID NO: 17 - protein, 482 aa, synthetic construct
  REGION 1..482: note = amino acid sequence of lightly M6P-glycosylated type hSGSH 2
RPRNALLLLADDGGFESGAYNNSAIATPHLDALARRSLLFRNAFTSVSSCSPSRASLLTGLPQHQNGMYGLHQDVHHFNSFDKVRSLPLLLSQAGVRTGIIGKKHVGPETVYPFDFAYTEENGSVLQVGRNITRIKLLVRKFLQTQDDRPFFLYVAFHDPHRCGHSQPQYGTFCEKFGNGESGMGRIPDWTPQAYDPLDVLVPYFVPNTPAARADLAAQYTTVGRMDQGVGLVLQELRDAGVLNDALVIFTSDNGIPFPSGRTNLYWPGTAEPLLVSSPEHPKRWGQVSEAYVSLLDLTPTILDWFSIPYPSYAIFGSKTIHLTGRSLLPALEAEPLWATVFGSQSHHEVTMSYPMRSVQHRHFRLVHNLNFKMPFPIDQDFYVSPTFQDLLNRTTAGQPTGWYKDLRHYYYRARWELYDRSRDPHETQNLATDPRFAQLLEMLRDQLAKWQWETHDPWVCAPDGVLEEKLSPQCQPLHNEL

SEQ ID NO: 18 - protein, 482 aa, synthetic construct
  REGION 1..482: note = amino acid sequence of lightly M6P-glycosylated type hSGSH 3
RPRNALLLLADDGGFESGAYNNSAIATPHLDALARRSLLFRNAFTSVSSCSPSRASLLTGLPQHQNGMYGLHQDVHHFNSFDKVRSLPLLLSQAGVRTGIIGKKHVGPETVYPFDFAYTEENGSVLQVGRNITRIKLLVRKFLQTQDDRPFFLYVAFHDPHRCGHSQPQYGTFCEKFGNGESGMGRIPDWTPQAYDPLDVLVPYFVPNTPAARADLAAQYTTVGRMDQGVGLVLQELRDAGVLQDALVIFTSDNGIPFPSGRTNLYWPGTAEPLLVSSPEHPKRWGQVSEAYVSLLDLTPTILDWFSIPYPSYAIFGSKTIHLTGRSLLPALEAEPLWATVFGSQSHHEVTMSYPMRSVQHRHFRLVHNLNFKMPFPIDQDFYVSPTFQDLLNRTTAGQPTGWYKDLRHYYYRARWELYDRSRDPHETQNLATDPRFAQLLEMLRDQLAKWQWETHDPWVCAPDGVLEEKLSPQCQPLHNEL

SEQ ID NO: 19 - protein, 883 aa, Homo sapiens
AHPGRPRAVPTQCDVPPNSRFDCAPDKAITQEQCEARGCCYIPAKQGLQGAQMGQPWCFFPPSYPSYKLENLSSSEMGYTATLTRTTPTFFPKDILTLRLDVMMETENRLHFTIKDPANRRYEVPLETPRVHSRAPSPLYSVEFSEEPFGVIVHRQLDGRVLLNTTVAPLFFADQFLQLSTSLPSQYITGLAEHLSPLMLSTSWTRITLWNRDLAPTPGANLYGSHPFYLALEDGGSAHGVFLLNSNAMDVVLQPSPALSWRSTGGILDVYIFLGPEPKSVVQQYLDVVGYPFMPPYWGLGFHLCRWGYSSTAITRQVVENMTRAHFPLDVQWNDLDYMDSRRDFTFNKDGFRDFPAMVQELHQGGRRYMMIVDPAISSSGPAGSYRPYDEGLRRGVFITNETGQPLIGKVWPGSTAFPDFTNPTALAWWEDMVAEFHDQVPFDGMWIDMNEPSNFIRGSEDGCPNNELENPPYVPGVVGGTLQAATICASSHQFLSTHYNLHNLYGLTEAIASHRALVKARGTRPFVISRSTFAGHGRYAGHWTGDVWSSWEQLASSVPEILQFNLLGVPLVGADVCGFLGNTSEELCVRWTQLGAFYPFMRNHNSLLSLPQEPYSFSEPAQQAMRKALTLRYALLPHLYTLFHQAHVAGETVARPLFLEFPKDSSTWTVDHQLLWGEALLITPVLQAGKAEVTGYFPLGTWYDLQTVPIEALGSLPPPPAAPREPAIHSEGQWVTLPAPLDTINVHLRAGYIIPLQGPGLTTTESRQQPMALAVALTKGGEARGELFWDDGESLEVLERGAYTQVIFLARNNTIVNELVRVTSEGAGLQLQKVTVLGVATAPQQVLSNGVPVSNFTYSPDTKVLDICVSLLMGEQFLVSWC

SEQ ID NO: 20 - DNA, 2652 bp, Homo sapiens
  source 1..2652: mol_type = genomic DNA
gctcaccccggtaggcctagggctgtccccacccagtgtgacgtcccccccaactctcgttttgattgcgcccccgataaggctatcacccaagaacaatgcgaagctcggggctgctgttacattcccgctaagcaaggtctccaaggtgcccagatgggccaaccttggtgtttttttccccccagctaccctagctacaagctggaaaacctcagctccagcgagatgggctacacagccacactcacacggacaacccccacctttttccctaaagacatcctcactttacggctcgatgtgatgatggagaccgaaaataggctccacttcaccatcaaggatcccgctaaccggcggtacgaggtgcctctcgagacccctcgtgtgcattctcgtgctcctagccctctgtacagcgtcgagttctccgaagagcctttcggagtgattgtccatcgtcagctggacggtcgtgttttactcaataccaccgtcgcccctctgttctttgctgaccagttcctccaactgagcacatctttaccctcccagtacattaccggtttagctgagcatttaagccctctcatgctctccacaagctggactcgtatcacactgtggaatcgtgacctcgcccctacacccggtgctaacctctacggaagccaccctttctacctcgctctcgaagacggcggcagcgcccatggcgtcttcctcctcaattccaacgctatggacgtcgtgctgcagcctagccccgctctcagctggaggtccaccggcggcattttagatgtctacatctttctgggccccgagcccaaatccgtcgtgcaacagtatttagacgtggtgggataccccttcatgcccccttattggggactcggcttccatctgtgtcggtggggctattccagcaccgccattacccggcaagttgtggagaatatgacccgggcccacttccctttagacgtgcagtggaatgatctggactacatggactcccggcgggactttacctttaacaaagacggctttcgggacttccccgccatggtgcaagaactgcaccaaggtggacggaggtacatgatgattgtggaccccgctatcagctccagcggacccgctggaagctaccggccctacgacgaaggactgcggcggggagtcttcatcaccaacgagactggtcaacctttaatcggcaaggtgtggcccggaagcacagccttccccgacttcaccaatcccacagctttagcttggtgggaggacatggtggccgagtttcacgaccaagttcctttcgacggcatgtggatcgacatgaacgagccttccaattttatccggggcagcgaggacggatgccctaataacgagctggagaaccctccctacgtccccggagtggtgggaggcacactgcaagccgctaccatctgcgccagctcccaccagtttctgtccacccactacaacctccacaatctgtacggactgaccgaggccattgcctcccatagggctttagtgaaagcccggggcacccggcctttcgtgatttctcgtagcacctttgccggccacggtcgttatgccggccattggaccggcgacgtctggagctcttgggagcagctggcttccagcgtgcccgaaatcctccagttcaatctcctcggagtgcctctggtgggcgccgatgtgtgtggctttctgggcaacaccagcgaggagctctgcgttcgttggacccagctcggagccttttatccctttatgcggaaccataatagcttattatctttacctcaagagccttattccttcagcgaacccgctcaacaagctatgcggaaggccctcactttaaggtacgctctgctccctcatttatacactttattccatcaagctcacgtcgctggcgagacagtggctaggcccctctttttagagttccccaaggactcctccacttggaccgtggatcatcagctgctgtggggagaggctttactgattacccccgtgctgcaagctggcaaggccgaggtgaccggctatttccctctgggcacttggtacgatttacagaccgtgcctattgaggctttaggctctttaccccctccccccgccgcccctagggagcccgctatccatagcgagggccaatgggtgacactgcccgctcctttagacaccatcaacgtccacttacgtgccggatacattatccccctccaaggtcccggtttaacaaccacagagtctcgtcagcaacctatggccctcgctgtggctctcacaaagggcggcgaggctcggggagagctgttttgggacgacggagaatctttagaagtgctcgagaggggcgcctacacccaagttatctttctggcccggaacaataccatcgtgaacgagctggttcgtgtgaccagcgaaggagccggtttacagctccaaaaggtgaccgtgctcggagtggctaccgcccctcagcaagttttatccaacggagtgcccgtgagcaactttacctacagccccgacacaaaggtcctcgacatctgtgtgtctttactgatgggcgaacagtttttagtgtcttggtgctga

SEQ ID NO: 21 - protein, 952 aa, Homo sapiens
MGVRHPPCSHRLLAVCALVSLATAALLGHILLHDFLLVPRELSGSSPVLEETHPAHQQGASRPGPRDAQAHPGRPRAVPTQCDVPPNSRFDCAPDKAITQEQCEARGCCYIPAKQGLQGAQMGQPWCFFPPSYPSYKLENLSSSEMGYTATLTRTTPTFFPKDILTLRLDVMMETENRLHFTIKDPANRRYEVPLETPRVHSRAPSPLYSVEFSEEPFGVIVHRQLDGRVLLNTTVAPLFFADQFLQLSTSLPSQYITGLAEHLSPLMLSTSWTRITLWNRDLAPTPGANLYGSHPFYLALEDGGSAHGVFLLNSNAMDVVLQPSPALSWRSTGGILDVYIFLGPEPKSVVQQYLDVVGYPFMPPYWGLGFHLCRWGYSSTAITRQVVENMTRAHFPLDVQWNDLDYMDSRRDFTFNKDGFRDFPAMVQELHQGGRRYMMIVDPAISSSGPAGSYRPYDEGLRRGVFITNETGQPLIGKVWPGSTAFPDFTNPTALAWWEDMVAEFHDQVPFDGMWIDMNEPSNFIRGSEDGCPNNELENPPYVPGVVGGTLQAATICASSHQFLSTHYNLHNLYGLTEAIASHRALVKARGTRPFVISRSTFAGHGRYAGHWTGDVWSSWEQLASSVPEILQFNLLGVPLVGADVCGFLGNTSEELCVRWTQLGAFYPFMRNHNSLLSLPQEPYSFSEPAQQAMRKALTLRYALLPHLYTLFHQAHVAGETVARPLFLEFPKDSSTWTVDHQLLWGEALLITPVLQAGKAEVTGYFPLGTWYDLQTVPIEALGSLPPPPAAPREPAIHSEGQWVTLPAPLDTINVHLRAGYIIPLQGPGLTTTESRQQPMALAVALTKGGEARGELFWDDGESLEVLERGAYTQVIFLARNNTIVNELVRVTSEGAGLQLQKVTVLGVATAPQQVLSNGVPVSNFTYSPDTKVLDICVSLLMGEQFLVSWC

SEQ ID NO: 22 - protein, 883 aa, synthetic construct
  REGION 1..883: note = amino acid sequence of lightly M6P-glycosylated type hGAA 1
AHPGRPRAVPTQCDVPPNSRFDCAPDKAITQEQCEARGCCYIPAKQGLQGAQMGQPWCFFPPSYPSYKLEQLSSSEMGYTATLTRTTPTFFPKDILTLRLDVMMETENRLHFTIKDPANRRYEVPLETPRVHSRAPSPLYSVEFSEEPFGVIVHRQLDGRVLLQTTVAPLFFADQFLQLSTSLPSQYITGLAEHLSPLMLSTSWTRITLWNRDLAPTPGANLYGSHPFYLALEDGGSAHGVFLLNSNAMDVVLQPSPALSWRSTGGILDVYIFLGPEPKSVVQQYLDVVGYPFMPPYWGLGFHLCRWGYSSTAITRQVVENMTRAHFPLDVQWNDLDYMDSRRDFTFNKDGFRDFPAMVQELHQGGRRYMMIVDPAISSSGPAGSYRPYDEGLRRGVFITQETGQPLIGKVWPGSTAFPDFTNPTALAWWEDMVAEFHDQVPFDGMWIDMNEPSNFIRGSEDGCPNNELENPPYVPGVVGGTLQAATICASSHQFLSTHYNLHNLYGLTEAIASHRALVKARGTRPFVISRSTFAGHGRYAGHWTGDVWSSWEQLASSVPEILQFNLLGVPLVGADVCGFLGNTSEELCVRWTQLGAFYPFMRNHNSLLSLPQEPYSFSEPAQQAMRKALTLRYALLPHLYTLFHQAHVAGETVARPLFLEFPKDSSTWTVDHQLLWGEALLITPVLQAGKAEVTGYFPLGTWYDLQTVPIEALGSLPPPPAAPREPAIHSEGQWVTLPAPLDTINVHLRAGYIIPLQGPGLTTTESRQQPMALAVALTKGGEARGELFWDDGESLEVLERGAYTQVIFLARNNTIVNELVRVTSEGAGLQLQKVTVLGVATAPQQVLSNGVPVSNFTYSPDTKVLDICVSLLMGEQFLVSWC

SEQ ID NO: 23 - protein, 883 aa, synthetic construct
  REGION 1..883: note = amino acid sequence of lightly M6P-glycosylated type hGAA 2
AHPGRPRAVPTQCDVPPNSRFDCAPDKAITQEQCEARGCCYIPAKQGLQGAQMGQPWCFFPPSYPSYKLENLASSEMGYTATLTRTTPTFFPKDILTLRLDVMMETENRLHFTIKDPANRRYEVPLETPRVHSRAPSPLYSVEFSEEPFGVIVHRQLDGRVLLNTAVAPLFFADQFLQLSTSLPSQYITGLAEHLSPLMLSTSWTRITLWNRDLAPTPGANLYGSHPFYLALEDGGSAHGVFLLNSNAMDVVLQPSPALSWRSTGGILDVYIFLGPEPKSVVQQYLDVVGYPFMPPYWGLGFHLCRWGYSSTAITRQVVENMTRAHFPLDVQWNDLDYMDSRRDFTFNKDGFRDFPAMVQELHQGGRRYMMIVDPAISSSGPAGSYRPYDEGLRRGVFITNEAGQPLIGKVWPGSTAFPDFTNPTALAWWEDMVAEFHDQVPFDGMWIDMNEPSNFIRGSEDGCPNNELENPPYVPGVVGGTLQAATICASSHQFLSTHYNLHNLYGLTEAIASHRALVKARGTRPFVISRSTFAGHGRYAGHWTGDVWSSWEQLASSVPEILQFNLLGVPLVGADVCGFLGNTSEELCVRWTQLGAFYPFMRNHNSLLSLPQEPYSFSEPAQQAMRKALTLRYALLPHLYTLFHQAHVAGETVARPLFLEFPKDSSTWTVDHQLLWGEALLITPVLQAGKAEVTGYFPLGTWYDLQTVPIEALGSLPPPPAAPREPAIHSEGQWVTLPAPLDTINVHLRAGYIIPLQGPGLTTTESRQQPMALAVALTKGGEARGELFWDDGESLEVLERGAYTQVIFLARNNTIVNELVRVTSEGAGLQLQKVTVLGVATAPQQVLSNGVPVSNFTYSPDTKVLDICVSLLMGEQFLVSWC

SEQ ID NO: 24 - protein, 883 aa, synthetic construct
  REGION 1..883: note = amino acid sequence of lightly M6P-glycosylated type hGAA 3
AHPGRPRAVPTQCDVPPNSRFDCAPDKAITQEQCEARGCCYIPAKQGLQGAQMGQPWCFFPPSYPSYKLEQLASSEMGYTATLTRTTPTFFPKDILTLRLDVMMETENRLHFTIKDPANRRYEVPLETPRVHSRAPSPLYSVEFSEEPFGVIVHRQLDGRVLLQTAVAPLFFADQFLQLSTSLPSQYITGLAEHLSPLMLSTSWTRITLWNRDLAPTPGANLYGSHPFYLALEDGGSAHGVFLLNSNAMDVVLQPSPALSWRSTGGILDVYIFLGPEPKSVVQQYLDVVGYPFMPPYWGLGFHLCRWGYSSTAITRQVVENMTRAHFPLDVQWNDLDYMDSRRDFTFNKDGFRDFPAMVQELHQGGRRYMMIVDPAISSSGPAGSYRPYDEGLRRGVFITQEAGQPLIGKVWPGSTAFPDFTNPTALAWWEDMVAEFHDQVPFDGMWIDMNEPSNFIRGSEDGCPNNELENPPYVPGVVGGTLQAATICASSHQFLSTHYNLHNLYGLTEAIASHRALVKARGTRPFVISRSTFAGHGRYAGHWTGDVWSSWEQLASSVPEILQFNLLGVPLVGADVCGFLGNTSEELCVRWTQLGAFYPFMRNHNSLLSLPQEPYSFSEPAQQAMRKALTLRYALLPHLYTLFHQAHVAGETVARPLFLEFPKDSSTWTVDHQLLWGEALLITPVLQAGKAEVTGYFPLGTWYDLQTVPIEALGSLPPPPAAPREPAIHSEGQWVTLPAPLDTINVHLRAGYIIPLQGPGLTTTESRQQPMALAVALTKGGEARGELFWDDGESLEVLERGAYTQVIFLARNNTIVNELVRVTSEGAGLQLQKVTVLGVATAPQQVLSNGVPVSNFTYSPDTKVLDICVSLLMGEQFLVSWC

SEQ ID NO: 25 - protein, 5 aa, synthetic construct
  REGION 1..5: note = amino acid sequence of an exemplified linker 1
GGGGS

SEQ ID NO: 26 - protein, 6 aa, synthetic construct
  REGION 1..6: note = amino acid sequence of an exemplified linker 2
GGGGGS

SEQ ID NO: 27 - protein, 5 aa, synthetic construct
  REGION 1..5: note = amino acid sequence of an exemplified linker 3
SGGGG

SEQ ID NO: 28 - protein, 760 aa, Homo sapiens
MMDQARSAFSNLFGGEPLSYTRFSLARQVDGDNSHVEMKLAVDEEENADNNTKANVTKPKRCSGSICYGTIAVIVFFLIGFMIGYLGYCKGVEPKTECERLAGTESPVREEPGEDFPAARRLYWDDLKRKLSEKLDSTDFTGTIKLLNENSYVPREAGSQKDENLALYVENQFREFKLSKVWRDQHFVKIQVKDSAQNSVIIVDKNGRLVYLVENPGGYVAYSKAATVTGKLVHANFGTKKDFEDLYTPVNGSIVIVRAGKITFAEKVANAESLNAIGVLIYMDQTKFPIVNAELSFFGHAHLGTGDPYTPGFPSFNHTQFPPSRSSGLPNIPVQTISRAAAEKLFGNMEGDCPSDWKTDSTCRMVTSESKNVKLTVSNVLKEIKILNIFGVIKGFVEPDHYVVVGAQRDAWGPGAAKSGVGTALLLKLAQMFSDMVLKDGFQPSRSIIFASWSAGDFGSVGATEWLEGYLSSLHLKAFTYINLDKAVLGTSNFKVSASPLLYTLIEKTMQNVKHPVTGQFLYQDSNWASKVEKLTLDNAAFPFLAYSGIPAVSFCFCEDTDYPYLGTTMDTYKELIERIPELNKVARAAAEVAGQFVIKLTHDVELNLDYERYNSQLLSFVRDLNQYRADIKEMGLSLQWLYSARGDFFRATSRLTTDFGNAEKTDRFVMKKLNDRVMRVEYHFLSPYVSPKESPFRHVFWGSGSHTLPALLENLKLRKQNNGAFNETLFRNQLALATWTIQGAANALSGDVWDIDNEF

SEQ ID NO: 29 - protein, 219 aa, synthetic construct
  REGION 1..219: note = amino acid sequence of the light chain of anti-hTfR antibody
DIVMTQTPLSLSVTPGQPASISCRSSQSLVHSNGNTYLHWYLQKPGQSPQLLIYKVSNRFSGVPDRFSGSGSGTDFTLKISRVEAEDVGVYYCSQSTHVPWTFGQGTKVEIKRTVAAPSVFIFPPSDEQLKSGTASVVCLLNNFYPREAKVQWKVDNALQSGNSQESVTEQDSKDSTYSLSSTLTLSKADYEKHKVYACEVTHQGLSSPVTKSFNRGEC

SEQ ID NO: 30 - protein, 448 aa, synthetic construct
  REGION 1..448: note = amino acid sequence of the heavy chain of anti-hTfR antibody
EVQLVQSGAEVKKPGESLKISCKGSGYSFMNYWLGWVRQMPGKGLEWMGDIYPGGDYPTYSEKFKVQVTISADKSISTAYLQLSSLKASDTAMYYCARSGNYDEVAYWGQGTLVTVSSASTKGPSVFPLAPSSKSTSGGTAALGCLVKDYFPEPVTVSWNSGALTSGVHTFPAVLQSSGLYSLSSVVTVPSSSLGTQTYICNVNHKPSNTKVDKKVEPKSCDKTHTCPPCPAPELLGGPSVFLFPPKPKDTLMISRTPEVTCVVVDVSHEDPEVKFNWYVDGVEVHNAKTKPREEQYNSTYRVVSVLTVLHQDWLNGKEYKCKVSNKALPAPIEKTISKAKGQPREPQVYTLPPSRDELTKNQVSLTCLVKGFYPSDIAVEWESNGQPENNYKTTPPVLDSDGSFFLYSKLTVDKSRWQQGNVFSCSVMHEALHNHYTQKSLSLSPGK

SEQ ID NO: 31 - protein, 226 aa, synthetic construct
  REGION 1..226: note = amino acid sequence of Fab heavy chain of anti-hTfR antibody
EVQLVQSGAEVKKPGESLKISCKGSGYSFMNYWLGWVRQMPGKGLEWMGDIYPGGDYPTYSEKFKVQVTISADKSISTAYLQLSSLKASDTAMYYCARSGNYDEVAYWGQGTLVTVSSASTKGPSVFPLAPSSKSTSGGTAALGCLVKDYFPEPVTVSWNSGALTSGVHTFPAVLQSSGLYSLSSVVTVPSSSLGTQTYICNVNHKPSNTKVDKKVEPKSCDKTHT

SEQ ID NO: 32 - DNA, 28 bp, synthetic construct
  misc_feature 1..28: note = pCI Insert F3 primer, synthetic sequence
  source 1..28: mol_type = other DNA
ctagcggcgcgcctcgcgaagcgctgca

SEQ ID NO: 33 - DNA, 28 bp, synthetic construct
  misc_feature 1..28: note = pCI Insert R3 primer, synthetic sequence
  source 1..28: mol_type = other DNA
ggcctgcagcgcttcgcgaggcgcgccg

SEQ ID NO: 34 - protein, 766 aa, synthetic construct
  REGION 1..766: note = amino acid sequence of fusion protein of wild type hIDS and Fabheavy chain of anti-hTfR antibody
EVQLVQSGAEVKKPGESLKISCKGSGYSFMNYWLGWVRQMPGKGLEWMGDIYPGGDYPTYSEKFKVQVTISADKSISTAYLQLSSLKASDTAMYYCARSGNYDEVAYWGQGTLVTVSSASTKGPSVFPLAPSSKSTSGGTAALGCLVKDYFPEPVTVSWNSGALTSGVHTFPAVLQSSGLYSLSSVVTVPSSSLGTQTYICNVNHKPSNTKVDKKVEPKSCDKTHTGGGGSGGGGSGGGGSSETQANSTTDALNVLLIIVDDLRPSLGCYGDKLVRSPNIDQLASHSLLFQNAFAQQAVCAPSRVSFLTGRRPDTTRLYDFNSYWRVHAGNFSTIPQYFKENGYVTMSVGKVFHPGISSNHTDDSPYSWSFPPYHPSSEKYENTKTCRGPDGELHANLLCPVDVLDVPEGTLPDKQSTEQAIQLLEKMKTSASPFFLAVGYHKPHIPFRYPKEFQKLYPLENITLAPDPEVPDGLPPVAYNPWMDIRQREDVQALNISVPYGPIPVDFQRKIRQSYFASVSYLDTQVGRLLSALDDLQLANSTIIAFTSDHGWALGEHGEWAKYSNFDVATHVPLIFYVPGRTASLPEAGEKLFPYLDPFDSASQLMEPGRQSMDLVELVSLFPTLAGLAGLQVPPRCPVPSFHVELCREGKNLLKHFRFRDLEEDPYLPGNPRELIAYSQYPRPSDIPQWNSDKPSLKDIKIMGYSIRTIDYRYTVWVGFNPDEFLANFSDIHAGELYFVDSDPLQDHNMYNDSQGGDLFQLLMP

SEQ ID NO: 35 - DNA, 2355 bp, synthetic construct
  misc_feature 1..2355: note = nucleic acid sequence coding fusion protein of wild type hIDS andFab heavy chain of anti-hTfR antibody, synthetic sequence
  source 1..2355: mol_type = other DNA
atgggttggagcctcatcttgctcttccttgtcgctgttgctacgcgagtcggcagcgaggtgcaactagtgcagtctggagcagaggtgaaaaagcccggggagtctctgaagatttcctgtaagggttctggatacagctttatgaactactggctgggatgggtgcgccagatgcccgggaaaggcctggagtggatgggggacatctaccccggcggagactaccctacatacagcgagaagttcaaggtccaggtcaccatctcagccgacaagtccatcagcaccgcctacctgcagttgagcagcctgaaggcctcggacaccgccatgtattactgtgcgagatcaggcaattacgacgaagtggcctactggggccaaggaaccctggtcaccgtctcctcagctagcaccaagggcccatcggtcttccccctggcaccctcctccaagagcacctctgggggcacagcggccctgggctgcctggtcaaggactacttccccgaaccggtgacggtgtcgtggaactcaggcgccctgaccagcggcgtgcacaccttcccggctgtcctacagtcctcaggactctactccctcagcagcgtggtgaccgtgccctccagcagcttgggcacccagacctacatctgcaacgtgaatcacaagcccagcaacaccaaggtggacaagaaagttgagccgaagagctgtgataagacgcatacgggtggcggagggtctggaggtggcggatcaggcggaggtggatcttccgaaacgcaggccaactcgaccacagatgctctgaacgttcttctcatcatcgtggatgacctgcgcccctccctgggctgttatggggataagctggtgaggtccccaaatattgaccaactggcatcccacagcctcctcttccagaatgcctttgcgcagcaagcagtgtgcgccccgagccgcgtttctttcctcactggcaggagacctgacaccacccgcctgtacgacttcaactcctactggagggtgcacgctggaaacttctccaccatcccccagtacttcaaggagaatggctatgtgaccatgtcggtgggaaaagtctttcaccctgggatatcttctaaccataccgatgattctccgtatagctggtcttttccaccttatcatccttcctctgagaagtatgaaaacactaagacatgtcgagggccagatggagaactccatgccaacctgctttgccctgtggatgtgctggatgttcccgagggcaccttgcctgacaaacagagcactgagcaagccatacagttgttggaaaagatgaaaacgtcagccagtcctttcttcctggccgttgggtatcataagccacacatccccttcagataccccaaggaatttcagaagttgtatcccttggagaacatcaccctggcccccgatcccgaggtccctgatggcctaccccctgtggcctacaacccctggatggacatcaggcaacgggaagacgtccaagccttaaacatcagtgtgccgtatggtccaattcctgtggactttcagcggaaaatccgccagagctactttgcctctgtgtcatatttggatacacaggtcggccgcctcttgagtgctttggacgatcttcagctggccaacagcaccatcattgcatttacctcggatcatgggtgggctctaggtgaacatggagaatgggccaaatacagcaattttgatgttgctacccatgttcccctgatattctatgttcctggaaggacggcttcacttccggaggcaggcgagaagcttttcccttacctcgacccttttgattccgcctcacagttgatggagccaggcaggcaatccatggaccttgtggaacttgtgtctctttttcccacgctggctggacttgcaggactgcaggttccacctcgctgccccgttccttcatttcacgttgagctgtgcagagaaggcaagaaccttctgaagcattttcgattccgtgacttggaagaagatccgtacctccctggtaatccccgtgaactgattgcctatagccagtatccccggccttcagacatccctcagtggaattctgacaagccgagtttaaaagatataaagatcatgggctattccatacgcaccatagactataggtatactgtgtgggttggcttcaatcctgatgaatttctagctaacttttctgacatccatgcaggggaactgtattttgtggattctgacccattgcaggatcacaatatgtataatgattcccaaggtggagaccttttccagttgttgatgcct

SEQ ID NO: 36 - DNA, 714 bp, synthetic construct
  misc_feature 1..714: note = nucleic acid sequence coding the light chain of anti-hTfRantibody, synthetic sequence
  source 1..714: mol_type = other DNA
atgggctggagctggattctgctgttcctcctgagcgtgacagcaggagtgcacagcgacatcgtgatgacccagactcccctgagcctgagcgtgacacctggccagcctgccagcatcagctgcagaagctctcagagcctggtgcacagcaacggcaacacctacctgcactggtatctgcagaagcccggccagagccctcagctgctgatctacaaggtgtccaacagattcagcggcgtgcccgacagattctccggcagcggctctggcaccgacttcaccctgaagatttccagagtggaagccgaggacgtgggcgtgtactactgcagccagagcacccacgtgccctggacattcggccagggcaccaaggtggaaatcaagagaaccgtggccgctcccagcgtgttcatcttcccacctagcgacgagcagctgaagtccggcacagcctctgtcgtgtgcctgctgaacaacttctacccccgcgaggccaaggtgcagtggaaggtggacaacgccctgcagagcggcaacagccaggaaagcgtgaccgagcaggactccaaggacagcacctacagcctgagcagcaccctgaccctgagcaaggccgactacgagaagcacaaggtgtacgcctgcgaagtgacccaccagggcctgtctagccccgtgaccaagagcttcaacagaggcgagtgc

SEQ ID NO: 37 - protein, 766 aa, synthetic construct
  REGION 1..766: note = amino acid sequence of fusion protein of muhIDS-1 and Fab heavychain of anti-hTfR antibody
EVQLVQSGAEVKKPGESLKISCKGSGYSFMNYWLGWVRQMPGKGLEWMGDIYPGGDYPTYSEKFKVQVTISADKSISTAYLQLSSLKASDTAMYYCARSGNYDEVAYWGQGTLVTVSSASTKGPSVFPLAPSSKSTSGGTAALGCLVKDYFPEPVTVSWNSGALTSGVHTFPAVLQSSGLYSLSSVVTVPSSSLGTQTYICNVNHKPSNTKVDKKVEPKSCDKTHTGGGGSGGGGSGGGGSSETQANSTTDALNVLLIIVDDLRPSLGCYGDKLVRSPNIDQLASHSLLFQNAFAQQAVCAPSRVSFLTGRRPDTTRLYDFNSYWRVHAGNFSTIPQYFKENGYVTMSVGKVFHPGISSNHTDDSPYSWSFPPYHPSSEKYENTKTCRGPDGELHANLLCPVDVLDVPEGTLPDKQSTEQAIQLLEKMKTSASPFFLAVGYHKPHIPFRYPKEFQKLYPLENIALAPDPEVPDGLPPVAYNPWMDIRQREDVQALNIAVPYGPIPVDFQRKIRQSYFASVSYLDTQVGRLLSALDDLQLANSTIIAFTSDHGWALGEHGEWAKYSNFDVATHVPLIFYVPGRTASLPEAGEKLFPYLDPFDSASQLMEPGRQSMDLVELVSLFPTLAGLAGLQVPPRCPVPSFHVELCREGKNLLKHFRFRDLEEDPYLPGNPRELIAYSQYPRPSDIPQWNSDKPSLKDIKIMGYSIRTIDYRYTVWVGFNPDEFLANFSDIHAGELYFVDSDPLQDHNMYNDSQGGDLFQLLMP

SEQ ID NO: 38 - DNA, 2355 bp, synthetic construct
  misc_feature 1..2355: note = nucleic acid sequence coding fusion protein of muhIDS-1 and Fabheavy chain of anti-hTfR antibody, synthetic sequence
  source 1..2355: mol_type = other DNA
atgggttggagcctcatcttgctcttccttgtcgctgttgctacgcgagtcggcagcgaggtgcaactagtgcagtctggagcagaggtgaaaaagcccggggagtctctgaagatttcctgtaagggttctggatacagctttatgaactactggctgggatgggtgcgccagatgcccgggaaaggcctggagtggatgggggacatctaccccggcggagactaccctacatacagcgagaagttcaaggtccaggtcaccatctcagccgacaagtccatcagcaccgcctacctgcagttgagcagcctgaaggcctcggacaccgccatgtattactgtgcgagatcaggcaattacgacgaagtggcctactggggccaaggaaccctggtcaccgtctcctcagctagcaccaagggcccatcggtcttccccctggcaccctcctccaagagcacctctgggggcacagcggccctgggctgcctggtcaaggactacttccccgaaccggtgacggtgtcgtggaactcaggcgccctgaccagcggcgtgcacaccttcccggctgtcctacagtcctcaggactctactccctcagcagcgtggtgaccgtgccctccagcagcttgggcacccagacctacatctgcaacgtgaatcacaagcccagcaacaccaaggtggacaagaaagttgagccgaagagctgtgataagacgcatacgggtggcggagggtctggaggtggcggatcaggcggaggtggatcttccgaaacgcaggccaactcgaccacagatgctctgaacgttcttctcatcatcgtggatgacctgcgcccctccctgggctgttatggggataagctggtgaggtccccaaatattgaccaactggcatcccacagcctcctcttccagaatgcctttgcgcagcaagcagtgtgcgccccgagccgcgtttctttcctcactggcaggagacctgacaccacccgcctgtacgacttcaactcctactggagggtgcacgctggaaacttctccaccatcccccagtacttcaaggagaatggctatgtgaccatgtcggtgggaaaagtctttcaccctgggatatcttctaaccataccgatgattctccgtatagctggtcttttccaccttatcatccttcctctgagaagtatgaaaacactaagacatgtcgagggccagatggagaactccatgccaacctgctttgccctgtggatgtgctggatgttcccgagggcaccttgcctgacaaacagagcactgagcaagccatacagttgttggaaaagatgaaaacgtcagccagtcctttcttcctggccgttgggtatcataagccacacatccccttcagataccccaaggaatttcagaagttgtatcccttggagaacatcgccctggcccccgatcccgaggtccctgatggcctaccccctgtggcctacaacccctggatggacatcaggcaacgggaagacgtccaagccttaaacatcgctgtgccgtatggtccaattcctgtggactttcagcggaaaatccgccagagctactttgcctctgtgtcatatttggatacacaggtcggccgcctcttgagtgctttggacgatcttcagctggccaacagcaccatcattgcatttacctcggatcatgggtgggctctaggtgaacatggagaatgggccaaatacagcaattttgatgttgctacccatgttcccctgatattctatgttcctggaaggacggcttcacttccggaggcaggcgagaagcttttcccttacctcgacccttttgattccgcctcacagttgatggagccaggcaggcaatccatggaccttgtggaacttgtgtctctttttcccacgctggctggacttgcaggactgcaggttccacctcgctgccccgttccttcatttcacgttgagctgtgcagagaaggcaagaaccttctgaagcattttcgattccgtgacttggaagaagatccgtacctccctggtaatccccgtgaactgattgcctatagccagtatccccggccttcagacatccctcagtggaattctgacaagccgagtttaaaagatataaagatcatgggctattccatacgcaccatagactataggtatactgtgtgggttggcttcaatcctgatgaatttctagctaacttttctgacatccatgcaggggaactgtattttgtggattctgacccattgcaggatcacaatatgtataatgattcccaaggtggagaccttttccagttgttgatgcct

SEQ ID NO: 39 - protein, 766 aa, synthetic construct
  REGION 1..766: note = amino acid sequence of fusion protein of muhIDS-2 and Fab heavychain of anti-hTfR antibody
EVQLVQSGAEVKKPGESLKISCKGSGYSFMNYWLGWVRQMPGKGLEWMGDIYPGGDYPTYSEKFKVQVTISADKSISTAYLQLSSLKASDTAMYYCARSGNYDEVAYWGQGTLVTVSSASTKGPSVFPLAPSSKSTSGGTAALGCLVKDYFPEPVTVSWNSGALTSGVHTFPAVLQSSGLYSLSSVVTVPSSSLGTQTYICNVNHKPSNTKVDKKVEPKSCDKTHTGGGGSGGGGSGGGGSSETQANSTTDALNVLLIIVDDLRPSLGCYGDKLVRSPNIDQLASHSLLFQNAFAQQAVCAPSRVSFLTGRRPDTTRLYDFNSYWRVHAGNFSTIPQYFKENGYVTMSVGKVFHPGISSNHTDDSPYSWSFPPYHPSSEKYENTKTCRGPDGELHANLLCPVDVLDVPEGTLPDKQSTEQAIQLLEKMKTSASPFFLAVGYHKPHIPFRYPKEFQKLYPLEQITLAPDPEVPDGLPPVAYNPWMDIRQREDVQALQISVPYGPIPVDFQRKIRQSYFASVSYLDTQVGRLLSALDDLQLANSTIIAFTSDHGWALGEHGEWAKYSNFDVATHVPLIFYVPGRTASLPEAGEKLFPYLDPFDSASQLMEPGRQSMDLVELVSLFPTLAGLAGLQVPPRCPVPSFHVELCREGKNLLKHFRFRDLEEDPYLPGNPRELIAYSQYPRPSDIPQWNSDKPSLKDIKIMGYSIRTIDYRYTVWVGFNPDEFLANFSDIHAGELYFVDSDPLQDHNMYNDSQGGDLFQLLMP

SEQ ID NO: 40 - DNA, 2355 bp, synthetic construct
  misc_feature 1..2355: note = nucleic acid sequence coding fusion protein of muhIDS-2 and Fabheavy chain of anti-hTfR antibody, synthetic sequence
  source 1..2355: mol_type = other DNA
atgggttggagcctcatcttgctcttccttgtcgctgttgctacgcgagtcggcagcgaggtgcaactagtgcagtctggagcagaggtgaaaaagcccggggagtctctgaagatttcctgtaagggttctggatacagctttatgaactactggctgggatgggtgcgccagatgcccgggaaaggcctggagtggatgggggacatctaccccggcggagactaccctacatacagcgagaagttcaaggtccaggtcaccatctcagccgacaagtccatcagcaccgcctacctgcagttgagcagcctgaaggcctcggacaccgccatgtattactgtgcgagatcaggcaattacgacgaagtggcctactggggccaaggaaccctggtcaccgtctcctcagctagcaccaagggcccatcggtcttccccctggcaccctcctccaagagcacctctgggggcacagcggccctgggctgcctggtcaaggactacttccccgaaccggtgacggtgtcgtggaactcaggcgccctgaccagcggcgtgcacaccttcccggctgtcctacagtcctcaggactctactccctcagcagcgtggtgaccgtgccctccagcagcttgggcacccagacctacatctgcaacgtgaatcacaagcccagcaacaccaaggtggacaagaaagttgagccgaagagctgtgataagacgcatacgggtggcggagggtctggaggtggcggatcaggcggaggtggatcttccgaaacgcaggccaactcgaccacagatgctctgaacgttcttctcatcatcgtggatgacctgcgcccctccctgggctgttatggggataagctggtgaggtccccaaatattgaccaactggcatcccacagcctcctcttccagaatgcctttgcgcagcaagcagtgtgcgccccgagccgcgtttctttcctcactggcaggagacctgacaccacccgcctgtacgacttcaactcctactggagggtgcacgctggaaacttctccaccatcccccagtacttcaaggagaatggctatgtgaccatgtcggtgggaaaagtctttcaccctgggatatcttctaaccataccgatgattctccgtatagctggtcttttccaccttatcatccttcctctgagaagtatgaaaacactaagacatgtcgagggccagatggagaactccatgccaacctgctttgccctgtggatgtgctggatgttcccgagggcaccttgcctgacaaacagagcactgagcaagccatacagttgttggaaaagatgaaaacgtcagccagtcctttcttcctggccgttgggtatcataagccacacatccccttcagataccccaaggaatttcagaagttgtatcccttggagcagatcaccctggcccccgatcccgaggtccctgatggcctaccccctgtggcctacaacccctggatggacatcaggcaacgggaagacgtccaagccttacagatcagtgtgccgtatggtccaattcctgtggactttcagcggaaaatccgccagagctactttgcctctgtgtcatatttggatacacaggtcggccgcctcttgagtgctttggacgatcttcagctggccaacagcaccatcattgcatttacctcggatcatgggtgggctctaggtgaacatggagaatgggccaaatacagcaattttgatgttgctacccatgttcccctgatattctatgttcctggaaggacggcttcacttccggaggcaggcgagaagcttttcccttacctcgacccttttgattccgcctcacagttgatggagccaggcaggcaatccatggaccttgtggaacttgtgtctctttttcccacgctggctggacttgcaggactgcaggttccacctcgctgccccgttccttcatttcacgttgagctgtgcagagaaggcaagaaccttctgaagcattttcgattccgtgacttggaagaagatccgtacctccctggtaatccccgtgaactgattgcctatagccagtatccccggccttcagacatccctcagtggaattctgacaagccgagtttaaaagatataaagatcatgggctattccatacgcaccatagactataggtatactgtgtgggttggcttcaatcctgatgaatttctagctaacttttctgacatccatgcaggggaactgtattttgtggattctgacccattgcaggatcacaatatgtataatgattcccaaggtggagaccttttccagttgttgatgcct

SEQ ID NO: 41 - protein, 2491 aa, Homo sapiens
MGAAAGRSPHLGPAPARRPQRSLLLLQLLLLVAAPGSTQAQAAPFPELCSYTWEAVDTKNNVLYKINICGSVDIVQCGPSSAVCMHDLKTRTYHSVGDSVLRSATRSLLEFNTTVSCDQQGTNHRVQSSIAFLCGKTLGTPEFVTATECVHYFEWRTTAACKKDIFKANKEVPCYVFDEELRKHDLNPLIKLSGAYLVDDSDPDTSLFINVCRDIDTLRDPGSQLRACPPGTAACLVRGHQAFDVGQPRDGLKLVRKDRLVLSYVREEAGKLDFCDGHSPAVTITFVCPSERREGTIPKLTAKSNCRYEIEWITEYACHRDYLESKTCSLSGEQQDVSIDLTPLAQSGGSSYISDGKEYLFYLNVCGETEIQFCNKKQAAVCQVKKSDTSQVKAAGRYHNQTLRYSDGDLTLIYFGGDECSSGFQRMSVINFECNKTAGNDGKGTPVFTGEVDCTYFFTWDTEYACVKEKEDLLCGATDGKKRYDLSALVRHAEPEQNWEAVDGSQTETEKKHFFINICHRVLQEGKARGCPEDAAVCAVDKNGSKNLGKFISSPMKEKGNIQLSYSDGDDCGHGKKIKTNITLVCKPGDLESAPVLRTSGEGGCFYEFEWHTAAACVLSKTEGENCTVFDSQAGFSFDLSPLTKKNGAYKVETKKYDFYINVCGPVSVSPCQPDSGACQVAKSDEKTWNLGLSNAKLSYYDGMIQLNYRGGTPYNNERHTPRATLITFLCDRDAGVGFPEYQEEDNSTYNFRWYTSYACPEEPLECVVTDPSTLEQYDLSSLAKSEGGLGGNWYAMDNSGEHVTWRKYYINVCRPLNPVPGCNRYASACQMKYEKDQGSFTEVVSISNLGMAKTGPVVEDSGSLLLEYVNGSACTTSDGRQTTYTTRIHLVCSRGRLNSHPIFSLNWECVVSFLWNTEAACPIQTTTDTDQACSIRDPNSGFVFNLNPLNSSQGYNVSGIGKIFMFNVCGTMPVCGTILGKPASGCEAETQTEELKNWKPARPVGIEKSLQLSTEGFITLTYKGPLSAKGTADAFIVRFVCNDDVYSGPLKFLHQDIDSGQGIRNTYFEFETALACVPSPVDCQVTDLAGNEYDLTGLSTVRKPWTAVDTSVDGRKRTFYLSVCNPLPYIPGCQGSAVGSCLVSEGNSWNLGVVQMSPQAAANGSLSIMYVNGDKCGNQRFSTRITFECAQISGSPAFQLQDGCEYVFIWRTVEACPVVRVEGDNCEVKDPRHGNLYDLKPLGLNDTIVSAGEYTYYFRVCGKLSSDVCPTSDKSKVVSSCQEKREPQGFHKVAGLLTQKLTYENGLLKMNFTGGDTCHKVYQRSTAIFFYCDRGTQRPVFLKETSDCSYLFEWRTQYACPPFDLTECSFKDGAGNSFDLSSLSRYSDNWEAITGTGDPEHYLINVCKSLAPQAGTEPCPPEAAACLLGGSKPVNLGRVRDGPQWRDGIIVLKYVDGDLCPDGIRKKSTTIRFTCSESQVNSRPMFISAVEDCEYTFAWPTATACPMKSNEHDDCQVTNPSTGHLFDLSSLSGRAGFTAAYSEKGLVYMSICGENENCPPGVGACFGQTRISVGKANKRLRYVDQVLQLVYKDGSPCPSKSGLSYKSVISFVCRPEARPTNRPMLISLDKQTCTLFFSWHTPLACEQATECSVRNGSSIVDLSPLIHRTGGYEAYDESEDDASDTNPDFYINICQPLNPMHGVPCPAGAAVCKVPIDGPPIDIGRVAGPPILNPIANEIYLNFESSTPCLADKHFNYTSLIAFHCKRGVSMGTPKLLRTSECDFVFEWETPVVCPDEVRMDGCTLTDEQLLYSFNLSSLSTSTFKVTRDSRTYSVGVCTFAVGPEQGGCKDGGVCLLSGTKGASFGRLQSMKLDYRHQDEAVVLSYVNGDRCPPETDDGVPCVFPFIFNGKSYEECIIESRAKLWCSTTADYDRDHEWGFCRHSNSYRTSSIIFKCDEDEDIGRPQVFSEVRGCDVTFEWKTKVVCPPKKLECKFVQKHKTYDLRLLSSLTGSWSLVHNGVSYYINLCQKIYKGPLGCSERASICRRTTTGDVQVLGLVHTQKLGVIGDKVVVTYSKGYPCGGNKTASSVIELTCTKTVGRPAFKRFDIDSCTYYFSWDSRAACAVKPQEVQMVNGTITNPINGKSFSLGDIYFKLFRASGDMRTNGDNYLYEIQLSSITSSRNPACSGANICQVKPNDQHFSRKVGTSDKTKYYLQDGDLDVVFASSSKCGKDKTKSVSSTIFFHCDPLVEDGIPEFSHETADCQYLFSWYTSAVCPLGVGFDSENPGDDGQMHKGLSERSQAVGAVLSLLLVALTCCLLALLLYKKERRETVISKLTTCCRRSSNVSYKYSKVNKEEETDENETEWLMEEIQLPPPRQGKEGQENGHITTKSVKALSSLHGDDQDSEDEVLTIPEVKVHSGRGAGAESSHPVRNAQSNALQEREDDRVGLVRGEKARKGKSSSAQQKTVSSTKLVSFHDDSDEDLLHI

SEQ ID NO: 42 - protein, 159 aa, synthetic construct
  REGION 1..159: note = amino acid sequence of domain 9 of hM6PR with His-tag
SAVVRVEGDNCEVKDPRHGNLYDLKPLGLNDTIVSAGEYTYYFRVCGKLSSDVCPTSDKSKVVSSCQEKREPQGFHKVAGLLTQKLTYENGLLKMNFTGGDTCHKVYQRSTAIFFYCDRGTQRPVFLKETSDCSYLFEWRTQYACPPFGSGAPHHHHHH